European Patent Application EP 4 578 867 A1, published July 2, 2025. Title: Cyclic peptide or salt thereof, and MDMX inhibitor. Applicant: FUJIFILM Corporation. Application WO. The sequence listing filed with the application follows.

SEQUENCE LISTING (1 sequence)

SEQ ID NO: 1 - protein, 15 aa, synthetic construct
  REGION 1..15: note = Description of Artificial Sequence: syntesized peptide
LTFAYWAQLAAAAAA